European Patent Application EP 4 163 304 A1, published April 12, 2023. Title: Droplet and manufacturing method thereof. Applicant: TOHOKU UNIVERSITY Tokushima University KWANSEI GAKUIN EDUCATIONAL FOUNDATION. The sequence listing filed with the application follows.

SEQUENCE LISTING (21 sequences)

SEQ ID NO: 1 - protein, 37 aa, Homo sapiens
PTIVEREPWDGRDGELPVEDDIDLSDVELDDLGKDEL

SEQ ID NO: 2 - protein, 37 aa, Mus musculus
PTITPREPWDGKDGELPVEDDIDLSDVELDDLEKDEL

SEQ ID NO: 3 - protein, 38 aa, Gallus gallus
PKIHAVEPWDGKDGELPVEDDIDLSDVDLDDIWDKDEL

SEQ ID NO: 4 - protein, 37 aa, Bos taurus
PTISTREPWDGKDGELPVEDDIDLSDVELDDLEKDEL

SEQ ID NO: 5 - protein, 37 aa, Oryctolagus cuniculus
PAISVRDPWDGQDGVLPVEDDIDLSDVELDDLEKDEL

SEQ ID NO: 6 - protein, 37 aa, Ictalurus punctatus
PKIHTVEAWDGKDGVLPVEDDIDLSDVDLDDLDKDEL

SEQ ID NO: 7 - protein, 37 aa, Danio rerio
PKINTVQAWDGKDGELPMEDDIDLSDVDLDDLEKDEL

SEQ ID NO: 8 - protein, 440 aa, Homo sapiens
MALLVLGLVSCTFFLAVNGLYSSSDDVIELTPSNFNREVIQSDSLWLVEFYAPWCGHCQRLTPEWKKAATALKDVVKVGAVDADKHHSLGGQYGVQGFPTIKIFGSNKNRPEDYQGGRTGEAIVDAALSALRQLVKDRLGGRSGGYSSGKQGRSDSSSKKDVIELTDDSFDKNVLDSEDVWMVEFYAPWCGHCKNLEPEWAAAASEVKEQTKGKVKLAAVDATVNQVLASRYGIRGFPTIKIFQKGESPVDYDGGRTRSDIVSRALDLFSDNAPPPELLEIINEDIAKRTCEEHQLCVVAVLPHILDTGAAGRNSYLEVLLKLADKYKKKMWGWLWTEAGAQSELETALGIGGFGYPAMAAINARKMKFALLKGSFSEQGINEFLRELSFGRGSTAPVGGGAFPTIVEREPWDGRDGELPVEDDIDLSDVELDDLGKDEL

SEQ ID NO: 9 - protein, 440 aa, Mus musculus
MARLVLGLVSCTFFLAVSGLYSSSDDVIELTPSNFNREVIQSDGLWLVEFYAPWCGHCQRLTPEWKKAATALKDVVKVGAVNADKHQSLGGQYGVQGFPTIKIFGANKNKPEDYQGGRTGEAIVDAALSALRQLVKDRLGGRSGGYSSGKQGRGDSSSKKDVVELTDDTFDKNVLDSEDVWMVEFYAPWCGHCKNLEPEWAAAATEVKEQTKGKVKLAAVDATVNQVLASRYGIKGFPTIKIFQKGESPVDYDGGRTRSDIVSRALDLFSDNAPPPELLEIINEDIAKKTCEEHQLCVVAVLPHILDTGAAGRNSYLEVLLKLADKYKKKMWGWLWTEAGAQYELENALGIGGFGYPAMAAINARKMKFALLKGSFSEQGINEFLRELSFGRGSTAPVGGGSFPTITPREPWDGKDGELPVEDDIDLSDVELDDLEKDEL

SEQ ID NO: 10 - protein, 447 aa, Gallus gallus
MGVRGTGGLWWGTVSCTLFLAVNGLYSASDDVIELTPTNFNKEVIQSESLWLVEFYAPWCGHCQRLTPEWKKAATALKGVVKVGAVDADKHQSLGGQYGVRGFPTIKIFGANKNKAEDYQGGRTSEAIVDAALSALRSLVKDRLSGRSGGYSSGRQSRESGGGDKKDVIELTDDSFDKNVINSDDVWMVEFYAPWCGHCKNLEPEWAAAATEVKEQTKGKVKLAAVDATVNQMLANRYGIRGFPTIKIFQKGEDPVDYDGGRTRSDITARALDLFSDNAPPPELLEIINEDVLKTTCDAHQLCIISVLPHILDTGASGRNSYLDVMLKMAEKYKKKMWGWLWTEAGAQSDLESSLGIGGFGYPAMAAINARKMKFALLKGSFSEQGINEFLRELSVGRGSTAPVGGGAFPKIHAVEPWDGKDGELPVEDDIDLSDVDLDDIWDKDEL

SEQ ID NO: 11 - protein, 453 aa, Bos taurus
RRRLECVAARALSMARLVLGLMSCTLFITVNGLYSSSDDVIELTPSNFNREVIQSDSLWLVEFYAPWCGHCQRLTPEWKKAATALKDVVKVGAVDADKHQSLGGQYGVQGFPTIKIFGSNKNKPEDYQGGRTGEAIVDAALSALRQLVKDRLGGRGSGYSSGKQGRGDSSSKKDVIELTDDNFDKNVLDSEDVWMVEFYAPWCGHCKNLEPEWAAAATEVKEQTKGKVKLAAVDATVNQVLASRYGIRGFPTIKIFQKGESPVDYDGGRTRSDIVSRALDLFSDNAPPPELLEIINEDVAKKTCEEHQLCVVAVLPHILDTGAAGRNSYLEVLLKLADKYKKKMWGWLWTEAGAQSELENALGIGGFGYPAMAAINARKMKFALLKGSFSEQGINEFLRELSFGRGSTAPVGGGAFPTISTREPWDGKDGELPVEDDIDLSDVELDDLEKDEL

SEQ ID NO: 12 - protein, 440 aa, Oryctolagus cuniculus
MARLGLGLVSCTFFLAVNGLYSSSDDVIELTPSNFNREVIQSDSLWLVEFYAPWCGHCQRLTPEWKKAASALKDVVKVGAVDADKHQALGGQYGVQGFPTIKIFGANKNRPEDYQGGRTGEAIVDAALSALRQLVKDRLGGRSGSHSSGRQGRGDSASKKDVIELTDDSFDENVLESDDIWMVEFYAPWCGHCKNLEPEWAAAATEVKEQTKGKVKLAAVDATVNQMLSSRYGIRGFPTIKIFQKGESPVDYDGGRTRSDIVSRALDLFSDNAPPPELLEIVNEDVAKRACEEHQLCIVAVLPHILDTGAAGRNSYLDVLLKLADKYKKKMWGWLWTEAGAQAELESALGIGGFGYPAMAAINARKMKFALLKGSFSEQGINEFLRELSFGRGSTAPVGGGVFPAISVRDPWDGQDGVLPVEDDIDLSDVELDDLEKDEL

SEQ ID NO: 13 - protein, 439 aa, Ictalurus punctatus
MRAFFGVLACSLTVLSVHGLYSASDDVIELNPSNFNREVLQSDSLWLVEFYAPWCGHCQSLVPEWKKAATALKGVVKVGAVDADQHKSLGGQYGVRGFPTIKIFGANKHKPEDYQGGRSSQAIVEAALNAARSLVKDRLSGKSGGSDYSRQSSGGGNKKDVVELTDDNFDRMVLDGDAVWMVEFFAPWCGHCKNLEPEWTAAATQVKEQTSGRVKLGAVDATVHQGLASRYGIKGFPTIKIFRKGEEPEDYQGGRTRSDIIARAIDLFSDNAPPPELLEILNEDILKKTCEDHQLCIIAVLPHILDTGAAGRNAYLEVMMKMAEKYKKKMWGWLWTESGAQMELEASLGIGGFGYPAMAAINARKMKFALLKGSFSETGIYEFLRDLSVGRGSTATITGGALPKIHTVEAWDGKDGVLPVEDDIDLSDVDLDDLDKDEL

SEQ ID NO: 14 - protein, 440 aa, Danio rerio
MRALLGVLACSLTVLSAYGLYTSSDDVVELNPSNFNREVIQSDSLWLVEFYAPWCGHCKSLAPEWKKAATALKGIVKVGAVDADQHNSLGGQYGVRGFPTIKIFGGNKHKPEDYQGGRTNQAIVDAALNALRSLVKDRLGGKTGGSDYSRQSGGGAGNKKDVVELTDDNFDRTVLESDDVWLVEFFAPWCGHCKNLEPEWTAAATEVKEQTKGKVKLAAVDATVHQGLASRFGIRGFPTIKVFRKGEEPEDYQGGRTRSDIVARALELYSDNIPAPELQEVLNEGILKKTCEDYQLCIIAVLPHILDTGASGRNSYLEVMKTMAEKYKKKMWGWLWTEAGAQMELEASLGIGGFGYPAMAAINSRKMKFALLKGSFSETGIHEFLRELSVGRGSTATVGGGALPKINTVQAWDGKDGELPMEDDIDLSDVDLDDLEKDEL

SEQ ID NO: 15 - protein, 55 aa, Homo sapiens
PEDYQGGRTGEAIVDAALSALRQLVKDRLGGRSGGYSSGKQGRSDSSSKKDVIEL

SEQ ID NO: 16 - protein, 55 aa, Mus musculus
PEDYQGGRTGEAIVDAALSALRQLVKDRLGGRSGGYSSGKQGRGDSSSKKDVVEL

SEQ ID NO: 17 - protein, 56 aa, Gallus gallus
AEDYQGGRTSEAIVDAALSALRSLVKDRLSGRSGGYSSGRQSRESGGGDKKDVIEL

SEQ ID NO: 18 - protein, 55 aa, Bos taurus
PEDYQGGRTGEAIVDAALSALRQLVKDRLGGRGSGYSSGKQGRGDSSSKKDVIEL

SEQ ID NO: 19 - protein, 55 aa, Oryctolagus cuniculus
PEDYQGGRTGEAIVDAALSALRQLVKDRLGGRSGSHSSGRQGRGDSASKKDVIEL

SEQ ID NO: 20 - protein, 54 aa, Ictalurus punctatus
PEDYQGGRSSQAIVEAALNAARSLVKDRLSGKSGGSDYSRQSSGGGNKKDVVEL

SEQ ID NO: 21 - protein, 55 aa, Danio rerio
PEDYQGGRTNQAIVDAALNALRSLVKDRLGGKTGGSDYSRQSGGGAGNKKDVVEL